European Patent Application EP 4 124 338 A1, published February 1, 2023. Title: Sigma-1 receptor modulator for use in the treatment of a pathology associated with WFS1 mutation. Applicant: Université de Montpellier Ecole Pratique des Hautes Etudes Institut National de la Santé et de la Recherche Médicale. The sequence listing filed with the application follows.

SEQUENCE LISTING (16 sequences)

SEQ ID NO: 1 - DNA, 20 bp, Artificial
  PCR primer WfsKO_wtF2
ttggcttgtatttgtcggcc

SEQ ID NO: 2 - DNA, 21 bp, Artificial
  PCR primer NeoR1
gaccgctatcaggacatagcg

SEQ ID NO: 3 - DNA, 20 bp, Artificial
  PCR primer WfsKO_uniR2
cccatcctgctctctgaacc

SEQ ID NO: 4 - DNA, 19 bp, Artificial
  Primer wfs1a forward
aatgaggagcagtgggttg

SEQ ID NO: 5 - DNA, 20 bp, Artificial
  Primer wfs1a reverse
ggcgaaggcaaacaaatcga

SEQ ID NO: 6 - DNA, 20 bp, Artificial
  Primer wfs1b forward
tctctccagcccaatacaga

SEQ ID NO: 7 - DNA, 20 bp, Artificial
  Primer wfs1b reverse
catctggatgttttactggc

SEQ ID NO: 8 - DNA, 22 bp, Artificial
  Primer s1r forward
atgagcaggctttctctaaggt

SEQ ID NO: 9 - DNA, 22 bp, Artificial
  Primer s1r reverse
tagtcgtcccctctttccattg

SEQ ID NO: 10 - DNA, 21 bp, Artificial
  Primer ncs1a forward
agccaaacaactcttcaggga

SEQ ID NO: 11 - DNA, 20 bp, Artificial
  Primer ncs1a reverse
gtccctgtctgtgtgtcagg

SEQ ID NO: 12 - DNA, 25 bp, Artificial
  Primer ncs1a forward
cccaattggaagaaagaaaattgca

SEQ ID NO: 13 - DNA, 20 bp, Artificial
  Primer ncs1b reverse
gggcttccatcaccaagaca

SEQ ID NO: 14 - DNA, 20 bp, Artificial
  Primer zef1a forward
ttctgttacctggcaaaggg

SEQ ID NO: 15 - DNA, 20 bp, Artificial
  Primer zef1a reverse
ttcagtttgtccaacaccca

SEQ ID NO: 16 - protein, 21 aa, Artificial
  Fragment of SIG-1R amino acids 142-161
KSEVFYPGETVVHGPGEATAV